European Patent Application EP 4 803 187 A1, published September 9, 2026. Title: CONTROLLED CELL-CELL INTERACTION ASSAY. Applicant: Singleron Biotechnologies Inc. The sequence listing filed with the application follows.

SEQUENCE LISTING (55 sequences)

SEQ ID NO: 1 - DNA, 11060 bp, synthetic construct
  source 1..11060: mol_type = other DNA
tacgaagagcaaaaaatacggcgattatttgatcgtcgcactttcaacagatgaatttaaccgtgaaaagggtaagaaaagttattttaactataacaaacgaaaatctcttttagaatctattagatatgttgatttagtcattccagaaaataattgggatcagaagataaatgatatgcatgaatatcatatcgatacttttgtcatgggcgatgactggaaaggaaaatttgatttcattaaggacgagggcgtagatgttgtttatctacctagaacccctgaaattagtacaagaaaaataaagagagatttgaaactttagtaagatacactttattacttataaagtgatattttctttttataatactttaaaagcatctttgcattttcagtagtatcatagcccttttcctttagcttttgacagtatgaatttgatcttagttcacggttgttagctataggtatttttatcttttggacccaatctttaggagaatctagtctttcaaaagaaatgttacttacaagatcattttctgaagaaattatattagatactacagcatctaatccggacgctgtcgtctctattaaagtataaggctgcccttcatataaagatggaagaagaaataaatccattgcattcagccatcccgaagtatcacttactgcaccagtgaagaatatatgtttacgcaaaaacgcatcactatcgacacgtttttttattttttcaaaattcacgccacttccaactaagactaaataataattatcgcctagctgtttaatcagatctagcaaaacaacctgatttttttgtctattaaattttcccacatttcccagcaaaatatcgtctttattaagtttaagtgtttttcgatagttttctcgcagactttcatcaaaatgaaaatgtgacaaatttattccatttcttataactaaaaattttttctgatgaaatagccacttgcccgcagcaatgttacatgctacacgtccattgactgttaaattaaagataggacgtaataatttatttatattcgtatgatcggcagttgtattatggctatgagctatacgaacttggattcctgcaatccatgcggccaaaagctcaactgacattgtagtactgttaccatttacatgaacaatatcatatttttctttttttaaaacttttattaatttccagaagtatatttgtggcgaattatctcgcatgggaagttcgattagtcttattccttttgaaattattctctttttaagggcttttttcactttattaggagcaataatagctacgtcttctccccacttagaaaaaagataactattatttaagatgaatgtagatataccattttcttctagattaacagtattaatcagtgcaatcttcatttttcacctaaagtttaaaatctacgagattatgtcgagttacccgttgatccttaggaggcaactctctccaattaccataatcatttactagcatttgttcataatatttagaaatcaagaaattgtgattttcaaatttatgatcctcagcttcatcaaaaaactttctgcaatacacatcttttttagcgtatgtacttggaaaaattctaacctttttagttttttctttatcatacttacacattatgtcaaaggccttattcctaatctttttagtattatttggaataagatatttaatcagaccagcaattattttcttttttccttttcgtgctttaacagataaatacttagccataaacatatgtcttaagaaaataaagctattaaattgttttttgtcttcggatttcttatcacttacattatcaacaggaaatatatctataaaaactccatgattaatattgtactcagccaaatatgactccttaaataaggtattgttaattcgaatcttatcaaacaaatataaatactctggatcagtgctcatatcttgataaaaatacttggaaggtaattctgttttacaaattaatttaaacttctccaagtcatcccttagcattgctatatccacatcatcccaaggaataaatacattatggcgaatcgctcccaataatgatccaccaattaaagtatatttaatagagtgttttctgcaaatctgatcaattactgtcagtgcttctaattctaaagagtgtatagcttttaattcattactcgataacacttttttttgcataaaaatcctgaattcttttaaaactaaattttattttttatgatgtttattgcatttttcaacattgaaatggcaattttattcttcaacaaaaccaaaattgcaccgtatataagaattgaagaatttactgaaaaaatcgttaccattatcattgaattccaactccattgacatagtaaacaaacacctactatcccaatacagccgataattgattctaaaagattttttaacgtttctttcttaaatataattggcttaataatatctctgcatgaataaccattcattatcattacactcaactctgccaacactgtgcttaatgaagtgccgtcatacgacattgtaggtatcaaaacgaaatttaaaattatattaattaccgccgttactaatgtatttcttaaaactttattttctcttttagctggaatcaatacacaatccgaaaaaatccaactaaaaattgagaaaataatcgcccacgtaataattcgaagtgaatttacagatggcaaaaacttttgaccagcaattattaaaacaacttctcgacttagcattaataggccaaccgatgcaggcaatactaacacacctaaagtgttaattactctagtcaatacgtcattatactctcttctccttctttgcccccatagcatagctaaccgaggtattgttactgttaaaacagcagaaagtagactttgtgctatctgatatatttttacagacgtactataaatcccaactgcataatcattcttcatcaatccaagaatagtattatctgaataaacatatatagttacagcaaccgaagaggcaaaaatagtcaatattggttttaaatgatattcccatctagtattcaaagttaaacgaatatgaataaaacttcgagcatgtacaaaattaaggaaatttgaaccaacactagccaacacggttatagcagcatatataagataatctgacggtctttttacaaaaataaataataaaattatcgataggattttaaaaattatacttctgatagtaatgtaggtataatcttcataaatcgtataaatccattcagtccctaaagtagtaaataaaatttggatactaaaaatcaatatacaagctacataattatttagatttttgaatattactaagctcaataataataatatgtatgcaattacggtagctaatatattgatactaaaaacttcgctagaaaactcctcaatttgttccttattatctctatactttgcaccctcacgaactgcatacgtagcaattcctaatccagcaattaatataaaatatccaatatatgtattagaaaaattataaattcctattccagagacagataaaacgcgagaaatatatgggaaagttactaatggaaatagtaaatttaaaacacttcttaatccatttaaaaaggcatttaatcccaaagattttttgctcatgactttcctttcttaagatttttgagtcttcttaaaatctttccaatcattccaatagttacaaataacggataacattttttgaaagcccaaatttcaatcttatatctggtattacaatccttcatatatatatcttgattcaaaaacttaattaaatctggatataattgaatttgagatttgtttaatctatgaaaaaaggaaatagcactaattagagtctctcttcttaattttgtacttagggaagaataatttgctttgaaaaaagtatacatttcataatgagataacgcagaatcctttaatttttttgttgaaagattatgagtcaatccattttcccttattcgatataaatatagagttgtattttctaatctaaaatgggtagctttatcatacaatttatatataatagccaagtcttcagtgtatatacgatcctcagggaatgctattttcttaaatagctctcttctaaaaattttattccatggaaaagtagcaaaacgctcatctaataacgtgcccatagcttgaaattttgagattcttttactatcgtctattctatttaaactgcaacttttatcgatattttttttctcttcaaagcgtaaataaccaaatattagtacatcaagattggagtaacaagttaggatcattttttttatgtattctaaactaccttttctaatagcatcatcactatctacaaaccatatccaatcaccagtactttttgataatccatagtttctagctctagatactcccgcattttccttatcaaaaatcctaatttgagaatatttagcttgatatctctcagcaatggttctactgttatcggtggaaccatcatttacaattattacttcaacattcttcaaatcattctgaattatactgtttaaacatatagcaatatagttttcaacattatacatcggaattattatacttattatcggctttttatctaccattttttagtttattcgctattttccatttcctcctaatattattttatacatcattcttaaataacttgaaccttaattaatatagaaagtattaaaatgaacttatgtttaataagcaaaacgaataatctctgtcttatagctaacttatcaattggataattttttatcacttcatttaagtcagcatttgaacaaatttctcgaacatttttaattattttccttattggcataaattctaactgagataatgatgatcgaacattaataaatagtgtcttagctaatcttagacgcgcttctgtaaatgacttattagccaaattcaatttactaagtttatctaccatatacataaagaaatatatacttttttcaaatctatctggtcggtaacttttagatagagattttggattagctctataataatatgcacttgaattaataattcttactccttttgcaaatttataatagtccgaatcccacacaatatcttcagaaatcagtttacgttccgaagcaaaaatgatcgaattttttttaataatcttacatgaatacagagaattccaaactgatggccgaaaagagttatgtttattagggctacttcctaacatactaacaaacaatttttgataaatactttcatgcctaaaaatagattcagtatattcacgagtataaagaacttcgccattatcctttactttggaatatcctccgattactgtatctatacttttaccatctagaccagcaactagtctttttattgcattctttcctaaataatcatcactatctacaaaagttacatactctccctttattctttctaatccatagtttctagtgaatcccaatcctgaatttgctttatgaaaagaataaacgaatgagtatgtttcagcataatcatcacatatttttccgctactatcagtagaaccatcatctatcaataatatttcaatattttgatatgtttgatcaactaatgactctatgcattttcttaaatatttttcaacgttataaatcggaaccacaattgaaactaatgaattcatttaatttccctttcagattatttcgccaatccatccacaattttctctagcttttcattaaattgcttattattactactttcaccgacatttttagttttagcaatttgatcataattatcaattgttgtttttaaatcatcaatatcgtatacaggaatgatattattcattctctctgcaatcaacttggtaaactcaacttgatgattatttacatgctcatgaaatttttcttgtcttggcactacaatcggaacttttccaaattgcaaagcctcgataaagctggaaggaccaccatgagtaattacaattcgtgcatcccttaacgcttgttgcatttcgtcaaaagacatcattttatgcgcttcgcagtttttaggaatataagtactgaaacctatttggataataaccttttctttaatatctccactagccactaaatcatcgactttttttataagacgattaaatggctgctcgtgtgtccctactgtaacaaagatcattaaaaaatactccctaaattaatagccttaggataaactttcttcatttcttcccattcgacaataaatcgatctgtaattggataaacaagtttcccagttaaagttggcttatcatagcgatcaaaaacctcaatatagactgtcttagcacccatcaatttaccaatataaaaaaatggaactgctactgcagctccactagaaataataacatcaggacgttctttacggagtactttaatagctaagaaagtatttttaattagattcttcagattacgattagtaggataatgacatccatacatcttctcacctttaagtttgcttcgagcatcttccttgtcaaaagttacccaaaaccgatctttattttgccaaaaaggttttaacatgtataaatgcgttaagtgtccaccactagacccaactaaacaaactttcataaaagatgtactccttaatacgctccattaggatgaataaccaccccaatagttttaataatcaactttaaatcttccaatattccagaatggttgatatacacgatatcaagccaagccatttcatcaaagtcagcttcgttacgtttagtaacttgccacaatcctgtacaacctggcataacaagcaatctctgcttatcatagtcagtatattcttctacctctgatggtaaaggtggacgtggtccaactagtgacatatcaccggttaggacattccataattgtggcaattcatcaagactgtacttacgaatagtatgaccaattttagtaattcttggatcatccttaatcttgaacatcgcaccattaatttcgttctgatcttccagttgatcaatcatttgatctgcattgacaaccattgaacgaaacttccacatcttaaatggtttttcatctttaccaattctctcttgtgaatagaatgctggtccaccgtcttcatgtcttatttttattattaaaaataaaaataatggagacagtagaatcaatccgaccgcactagcaataatatcaaacaatctcttcaatgcgtgataaacataccgcccatgcactttgaccggattaacttttagtttctccattaccatcattttttctcttaccctcaatgtcgctaatgccacaaatctgcagatttgcagattaaaatagccagaattttttctttttgccaagtggctgccaatctagctgcacattgtccccatttacaaatgcgcgagcattatcttcatattgctgagcaagatcactcctgaattccttgctcagcttttttaatgcttcactatattgatattgtctctttggcaaatcgtgcgcatccgaagcgaagcaggcacattggcctgctttgataaacttgcgtgacatttcttcaatttttttgccaaaggttcccatgtaagaactagcagtaatttgcactaagcatccctgctcaattaattcttgcaagatagttggctcttccagaatcttcttgttacgctctgggtgcaccacaattggtgtaatcccgcgctgcattaattcaaagaccatatctcgcgtataagctggtacatcgtcacttggaaattccaagagcatgtattgtccatccacatctaagaaaagaatatcgtcatcatctaatgccttaggcaagtctccagaaattctgacctcttgcccaggaaacaccgttaacggaatcttggcatcgtctaacatatcctgaaagttttctgttaaacgaataacgtctttcttatgattgatatacttgccattaagcatgtgcggcgtgcaaactgcatgagttaccccatccgcaactgcttctctagctaacttgattgatgtttgccaatctttggcaccatcatcgacgcccggcaagatatggcagtgaatatcaactaaaaccatttactttttcaacctagaaaatattccttttttcttctttgcgtcttcttcgccgtagccatatccataaccgtagccatatccataaccatagccggcattatcagaactaatatcgttcataatgaagcctaataccttggccttagagaagttaagcatttcaacagcacgtttaatggcagccttttgtgttttaccttgacgtactactaagataatgccgtctaagcgacgagctaattcttgcgtatcagatacttcaatcactggtgccaagtcgatgattaccatgtcatagtgatcttcaactaagctgatgaagtcttgcattctcttagatccaatcaattctgatgggttaggttgtgtaggaccagcaggtaagattgctaagtcagcaatcccactgtcttggacaacttcatctagatctacttcttttgcagtagaagagataactgtacttaatcctacatgattgcttaagttaaatgttctgtgaacagtaggacgacgtaagtcggcatcaatcaacaataccttatggcccgcttgagcataggttacagcaacgtttgcagcaacggctgacttaccttcactgatgctagcagaagtaaaagcaacagatttgatatcatggtcaactgccatgaagttaatgttggtacgaatggtacggaactgttcagttactggactcttaggatcagcaacagtaattaacttagcaccctttttaatggcttcatctgtaccacgttttttcttaaaaagtgacatcagttacctcctatactctgcgtctcttgcgttgttcacgcttagcagctggcttattattattattcttaatcaacttaaatgatgaagatacatggaagtgagatacatatcctaagttggtcaaacccaaatcttgagttaagtaagtatcatcacgaacagtggtattagtcatttcacgaattaagatcactgcaaaggttaatactaaaccaataacaaatcctgctaaagtaaacatcttaacgttaggtgatgattgaacaccattagtagctgatgcaacgatcgtaacgttatcgatattcatgatattaggaatttgatctctgaatgatctagcaactgcattagcttcagccttagccttttcaggagtatcagccgtagcagaaactgagaatacctgtgattgttgttgcgtagcaactgaaacactcttagctaattgcgcagctgaaacgctatatgccttaccgtcacgtttaatgactgctggttgagcctttctcaccaagacttttctaccattatcagtagttttgtacttagctggcttagccttcttaaccactctaactgggttagtcaaacgatcagaagcatccttcaagattacatgactagttacaatatctttataggtattaactaactgcatgttagcttgttgggttatatatgctgtattaggatcattcttattggatttttggttaactaagatttgtgcactagaagtatactttggtgaaatgacaaagttagcaattccccaacctactaatgttaatccaatactccaaagaatcaatgcccagatatgtctgcgacaaagttgaagcaattgagtaagatcaattgtattatcagtttgcttttgttcttgttccatctgtctttcctttaattatgattcataacgtaacttgctttattagcagctaccttagtctttggcaattctaaagcatccctaatcttatcagatactctttgtctttcttccttacttacaacttcgatttccatcaagccaaacttaggattcatagtttgcttacttacaccttgagcatggtcttggctcaagttatcagtggccttgcggtaatccataccaatcttgtacatttggttcatggtcaagtcagtctgcatttcatcagaaattgaattcaagaaattagaattcaacaaagttgttggtgaaacagacttcttaagaagcgccataattactcggcggtcacgatcttgacgaccgtagtcttgacgtggatctccgtgacgaagttgagcaaaggctaatgcttttttaccattcatatgataagtcttgccttcttcgaagtggtagcccatattattgaacgtaagtggtgaagttacatctataccaccgacttgatcgattgccttcttcaagccgcccatgttaatcatgatgtagccgtcaattggcacgctgtagtacttatccagcgtcttgatcgtctcgctaacgccgcccagcgtgtaagctgagttcatcttcgttaccccatattctgggtaatctgggaagattgcgttagagtcacgcggaatagatacaatggtagtcgtattcttcttagggttgatggacatcatcatcatggtatccgtccggcccttccagtgacgacccatcgcaccagtatcgatacccaataacaagatgttaattggtttcttttcatttaacaaattatcaagagtccgacccttgttgctcttcgtattcttagcaacgggggtgtacatgttttgcgttgtactacgcaggttcttgtaaaccatgccgcaaacaaaaagaccaatgaccacgacaattcctagcacaatccaaaaaccacgccaaaattttctgtgatgatgacgatggtgatggtgatgtcgacgcatcggctttttatcttgttgattcttttctaccatattaatcccctcaatatattatagaccttt

SEQ ID NO: 2 - DNA, 300 bp, synthetic construct
  source 1..300: mol_type = other DNA
ttgatcgtcgcactttcaacagatgaatttaaccgtgaaaagggtaagaaaagttattttaactataacaaacgaaaatctcttttagaatctattagatatgttgatttagtcattccagaaaataattgggatcagaagataaatgatatgcatgaatatcatatcgatacttttgtcatgggcgatgactggaaaggaaaatttgatttcattaaggacgagggcgtagatgttgtttatctacctagaacccctgaaattagtacaagaaaaataaagagagatttgaaactttag

SEQ ID NO: 3 - DNA, 1092 bp, synthetic construct
  source 1..1092: mol_type = other DNA
atgaagattgcactgattaatactgttaatctagaagaaaatggtatatctacattcatcttaaataatagttatcttttttctaagtggggagaagacgtagctattattgctcctaataaagtgaaaaaagcccttaaaaagagaataatttcaaaaggaataagactaatcgaacttcccatgcgagataattcgccacaaatatacttctggaaattaataaaagttttaaaaaaagaaaaatatgatattgttcatgtaaatggtaacagtactacaatgtcagttgagcttttggccgcatggattgcaggaatccaagttcgtatagctcatagccataatacaactgccgatcatacgaatataaataaattattacgtcctatctttaatttaacagtcaatggacgtgtagcatgtaacattgctgcgggcaagtggctatttcatcagaaaaaatttttagttataagaaatggaataaatttgtcacattttcattttgatgaaagtctgcgagaaaactatcgaaaaacacttaaacttaataaagacgatattttgctgggaaatgtgggaaaatttaatagacaaaaaaatcaggttgttttgctagatctgattaaacagctaggcgataattattatttagtcttagttggaagtggcgtgaattttgaaaaaataaaaaaacgtgtcgatagtgatgcgtttttgcgtaaacatatattcttcactggtgcagtaagtgatacttcgggatggctgaatgcaatggatttatttcttcttccatctttatatgaagggcagccttatactttaatagagacgacagcgtccggattagatgctgtagtatctaatataatttcttcagaaaatgatcttgtaagtaacatttcttttgaaagactagattctcctaaagattgggtccaaaagataaaaatacctatagctaacaaccgtgaactaagatcaaattcatactgtcaaaagctaaaggaaaagggctatgatactactgaaaatgcaaagatgcttttaaagtattataaaaagaaaatatcactttataagtaa

SEQ ID NO: 4 - DNA, 816 bp, synthetic construct
  source 1..816: mol_type = other DNA
atgcaaaaaaaagtgttatcgagtaatgaattaaaagctatacactctttagaattagaagcactgacagtaattgatcagatttgcagaaaacactctattaaatatactttaattggtggatcattattgggagcgattcgccataatgtatttattccttgggatgatgtggatatagcaatgctaagggatgacttggagaagtttaaattaatttgtaaaacagaattaccttccaagtatttttatcaagatatgagcactgatccagagtatttatatttgtttgataagattcgaattaacaataccttatttaaggagtcatatttggctgagtacaatattaatcatggagtttttatagatatatttcctgttgataatgtaagtgataagaaatccgaagacaaaaaacaatttaatagctttattttcttaagacatatgtttatggctaagtatttatctgttaaagcacgaaaaggaaaaaagaaaataattgctggtctgattaaatatcttattccaaataatactaaaaagattaggaataaggcctttgacataatgtgtaagtatgataaagaaaaaactaaaaaggttagaatttttccaagtacatacgctaaaaaagatgtgtattgcagaaagttttttgatgaagctgaggatcataaatttgaaaatcacaatttcttgatttctaaatattatgaacaaatgctagtaaatgattatggtaattggagagagttgcctcctaaggatcaacgggtaactcgacataatctcgtagattttaaactttag

SEQ ID NO: 5 - DNA, 1464 bp, synthetic construct
  source 1..1464: mol_type = other DNA
atgagcaaaaaatctttgggattaaatgcctttttaaatggattaagaagtgttttaaatttactatttccattagtaactttcccatatatttctcgcgttttatctgtctctggaataggaatttataatttttctaatacatatattggatattttatattaattgctggattaggaattgctacgtatgcagttcgtgagggtgcaaagtatagagataataaggaacaaattgaggagttttctagcgaagtttttagtatcaatatattagctaccgtaattgcatacatattattattattgagcttagtaatattcaaaaatctaaataattatgtagcttgtatattgatttttagtatccaaattttatttactactttagggactgaatggatttatacgatttatgaagattatacctacattactatcagaagtataatttttaaaatcctatcgataattttattatttatttttgtaaaaagaccgtcagattatcttatatatgctgctataaccgtgttggctagtgttggttcaaatttccttaattttgtacatgctcgaagttttattcatattcgtttaactttgaatactagatgggaatatcatttaaaaccaatattgactatttttgcctcttcggttgctgtaactatatatgtttattcagataatactattcttggattgatgaagaatgattatgcagttgggatttatagtacgtctgtaaaaatatatcagatagcacaaagtctactttctgctgttttaacagtaacaatacctcggttagctatgctatgggggcaaagaaggagaagagagtataatgacgtattgactagagtaattaacactttaggtgtgttagtattgcctgcatcggttggcctattaatgctaagtcgagaagttgttttaataattgctggtcaaaagtttttgccatctgtaaattcacttcgaattattacgtgggcgattattttctcaatttttagttggattttttcggattgtgtattgattccagctaaaagagaaaataaagttttaagaaatacattagtaacggcggtaattaatataattttaaatttcgttttgatacctacaatgtcgtatgacggcacttcattaagcacagtgttggcagagttgagtgtaatgataatgaatggttattcatgcagagatattattaagccaattatatttaagaaagaaacgttaaaaaatcttttagaatcaattatcggctgtattgggatagtaggtgtttgtttactatgtcaatggagttggaattcaatgataatggtaacgattttttcagtaaattcttcaattcttatatacggtgcaattttggttttgttgaagaataaaattgccatttcaatgttgaaaaatgcaataaacatcataaaaaataaaatttag

SEQ ID NO: 6 - DNA, 1002 bp, synthetic construct
  source 1..1002: mol_type = other DNA
atggtagataaaaagccgataataagtataataattccgatgtataatgttgaaaactatattgctatatgtttaaacagtataattcagaatgatttgaagaatgttgaagtaataattgtaaatgatggttccaccgataacagtagaaccattgctgagagatatcaagctaaatattctcaaattaggatttttgataaggaaaatgcgggagtatctagagctagaaactatggattatcaaaaagtactggtgattggatatggtttgtagatagtgatgatgctattagaaaaggtagtttagaatacataaaaaaaatgatcctaacttgttactccaatcttgatgtactaatatttggttatttacgctttgaagagaaaaaaaatatcgataaaagttgcagtttaaatagaatagacgatagtaaaagaatctcaaaatttcaagctatgggcacgttattagatgagcgttttgctacttttccatggaataaaatttttagaagagagctatttaagaaaatagcattccctgaggatcgtatatacactgaagacttggctattatatataaattgtatgataaagctacccattttagattagaaaatacaactctatatttatatcgaataagggaaaatggattgactcataatctttcaacaaaaaaattaaaggattctgcgttatctcattatgaaatgtatacttttttcaaagcaaattattcttccctaagtacaaaattaagaagagagactctaattagtgctatttccttttttcatagattaaacaaatctcaaattcaattatatccagatttaattaagtttttgaatcaagatatatatatgaaggattgtaataccagatataagattgaaatttgggctttcaaaaaatgttatccgttatttgtaactattggaatgattggaaagattttaagaagactcaaaaatcttaagaaaggaaagtcatga

SEQ ID NO: 7 - DNA, 1026 bp, synthetic construct
  source 1..1026: mol_type = other DNA
atgaattcattagtttcaattgtggttccgatttataacgttgaaaaatatttaagaaaatgcatagagtcattagttgatcaaacatatcaaaatattgaaatattattgatagatgatggttctactgatagtagcggaaaaatatgtgatgattatgctgaaacatactcattcgtttattcttttcataaagcaaattcaggattgggattcactagaaactatggattagaaagaataaagggagagtatgtaacttttgtagatagtgatgattatttaggaaagaatgcaataaaaagactagttgctggtctagatggtaaaagtatagatacagtaatcggaggatattccaaagtaaaggataatggcgaagttctttatactcgtgaatatactgaatctatttttaggcatgaaagtatttatcaaaaattgtttgttagtatgttaggaagtagccctaataaacataactcttttcggccatcagtttggaattctctgtattcatgtaagattattaaaaaaaattcgatcatttttgcttcggaacgtaaactgatttctgaagatattgtgtgggattcggactattataaatttgcaaaaggagtaagaattattaattcaagtgcatattattatagagctaatccaaaatctctatctaaaagttaccgaccagatagatttgaaaaaagtatatatttctttatgtatatggtagataaacttagtaaattgaatttggctaataagtcatttacagaagcgcgtctaagattagctaagacactatttattaatgttcgatcatcattatctcagttagaatttatgccaataaggaaaataattaaaaatgttcgagaaatttgttcaaatgctgacttaaatgaagtgataaaaaattatccaattgataagttagctataagacagagattattcgttttgcttattaaacataagttcattttaatactttctatattaattaaggttcaagttatttaa

SEQ ID NO: 8 - DNA, 498 bp, synthetic construct
  source 1..498: mol_type = other DNA
atgatctttgttacagtagggacacacgagcagccatttaatcgtcttataaaaaaagtcgatgatttagtggctagtggagatattaaagaaaaggttattatccaaataggtttcagtacttatattcctaaaaactgcgaagcgcataaaatgatgtcttttgacgaaatgcaacaagcgttaagggatgcacgaattgtaattactcatggtggtccttccagctttatcgaggctttgcaatttggaaaagttccgattgtagtgccaagacaagaaaaatttcatgagcatgtaaataatcatcaagttgagtttaccaagttgattgcagagagaatgaataatatcattcctgtatacgatattgatgatttaaaaacaacaattgataattatgatcaaattgctaaaactaaaaatgtcggtgaaagtagtaataataagcaatttaatgaaaagctagagaaaattgtggatggattggcgaaataa

SEQ ID NO: 9 - DNA, 450 bp, synthetic construct
  source 1..450: mol_type = other DNA
atgaaagtttgtttagttgggtctagtggtggacacttaacgcatttatacatgttaaaacctttttggcaaaataaagatcggttttgggtaacttttgacaaggaagatgctcgaagcaaacttaaaggtgagaagatgtatggatgtcattatcctactaatcgtaatctgaagaatctaattaaaaatactttcttagctattaaagtactccgtaaagaacgtcctgatgttattatttctagtggagctgcagtagcagttccatttttttatattggtaaattgatgggtgctaagacagtctatattgaggtttttgatcgctatgataagccaactttaactgggaaacttgtttatccaattacagatcgatttattgtcgaatgggaagaaatgaagaaagtttatcctaaggctattaatttagggagtattttttaa

SEQ ID NO: 10 - DNA, 651 bp, synthetic construct
  source 1..651: mol_type = other DNA
atggtaatggagaaactaaaagttaatccggtcaaagtgcatgggcggtatgtttatcacgcattgaagagattgtttgatattattgctagtgcggtcggattgattctactgtctccattatttttatttttaataataaaaataagacatgaagacggtggaccagcattctattcacaagagagaattggtaaagatgaaaaaccatttaagatgtggaagtttcgttcaatggttgtcaatgcagatcaaatgattgatcaactggaagatcagaacgaaattaatggtgcgatgttcaagattaaggatgatccaagaattactaaaattggtcatactattcgtaagtacagtcttgatgaattgccacaattatggaatgtcctaaccggtgatatgtcactagttggaccacgtccacctttaccatcagaggtagaagaatatactgactatgataagcagagattgcttgttatgccaggttgtacaggattgtggcaagttactaaacgtaacgaagctgactttgatgaaatggcttggcttgatatcgtgtatatcaaccattctggaatattggaagatttaaagttgattattaaaactattggggtggttattcatcctaatggagcgtattaa

SEQ ID NO: 11 - DNA, 771 bp, synthetic construct
  source 1..771: mol_type = other DNA
atggttttagttgatattcactgccatatcttgccgggcgtcgatgatggtgccaaagattggcaaacatcaatcaagttagctagagaagcagttgcggatggggtaactcatgcagtttgcacgccgcacatgcttaatggcaagtatatcaatcataagaaagacgttattcgtttaacagaaaactttcaggatatgttagacgatgccaagattccgttaacggtgtttcctgggcaagaggtcagaatttctggagacttgcctaaggcattagatgatgacgatattcttttcttagatgtggatggacaatacatgctcttggaatttccaagtgacgatgtaccagcttatacgcgagatatggtctttgaattaatgcagcgcgggattacaccaattgtggtgcacccagagcgtaacaagaagattctggaagagccaactatcttgcaagaattaattgagcagggatgcttagtgcaaattactgctagttcttacatgggaacctttggcaaaaaaattgaagaaatgtcacgcaagtttatcaaagcaggccaatgtgcctgcttcgcttcggatgcgcacgatttgccaaagagacaatatcaatatagtgaagcattaaaaaagctgagcaaggaattcaggagtgatcttgctcagcaatatgaagataatgctcgcgcatttgtaaatggggacaatgtgcagctagattggcagccacttggcaaaaagaaaaaattctggctattttaa

SEQ ID NO: 12 - DNA, 786 bp, synthetic construct
  source 1..786: mol_type = other DNA
atgtcactttttaagaaaaaacgtggtacagatgaagccattaaaaagggtgctaagttaattactgttgctgatcctaagagtccagtaactgaacagttccgtaccattcgtaccaacattaacttcatggcagttgaccatgatatcaaatctgttgcttttacttctgctagcatcagtgaaggtaagtcagccgttgctgcaaacgttgctgtaacctatgctcaagcgggccataaggtattgttgattgatgccgacttacgtcgtcctactgttcacagaacatttaacttaagcaatcatgtaggattaagtacagttatctcttctactgcaaaagaagtagatctagatgaagttgtccaagacagtgggattgctgacttagcaatcttacctgctggtcctacacaacctaacccatcagaattgattggatctaagagaatgcaagacttcatcagcttagttgaagatcactatgacatggtaatcatcgacttggcaccagtgattgaagtatctgatacgcaagaattagctcgtcgcttagacggcattatcttagtagtacgtcaaggtaaaacacaaaaggctgccattaaacgtgctgttgaaatgcttaacttctctaaggccaaggtattaggcttcattatgaacgatattagttctgataatgccggctatggttatggatatggctacggttatggatatggctacggcgaagaagacgcaaagaagaaaaaaggaatattttctaggttgaaaaagtaa

SEQ ID NO: 13 - DNA, 1056 bp, synthetic construct
  source 1..1056: mol_type = other DNA
atggtagaaaagaatcaacaagataaaaagccgatgcgtcgacatcaccatcaccatcgtcatcatcacagaaaattttggcgtggtttttggattgtgctaggaattgtcgtggtcattggtctttttgtttgcggcatggtttacaagaacctgcgtagtacaacgcaaaacatgtacacccccgttgctaagaatacgaagagcaacaagggtcggactcttgataatttgttaaatgaaaagaaaccaattaacatcttgttattgggtatcgatactggtgcgatgggtcgtcactggaagggccggacggataccatgatgatgatgtccatcaaccctaagaagaatacgactaccattgtatctattccgcgtgactctaacgcaatcttcccagattacccagaatatggggtaacgaagatgaactcagcttacacgctgggcggcgttagcgagacgatcaagacgctggataagtactacagcgtgccaattgacggctacatcatgattaacatgggcggcttgaagaaggcaatcgatcaagtcggtggtatagatgtaacttcaccacttacgttcaataatatgggctaccacttcgaagaaggcaagacttatcatatgaatggtaaaaaagcattagcctttgctcaacttcgtcacggagatccacgtcaagactacggtcgtcaagatcgtgaccgccgagtaattatggcgcttcttaagaagtctgtttcaccaacaactttgttgaattctaatttcttgaattcaatttctgatgaaatgcagactgacttgaccatgaaccaaatgtacaagattggtatggattaccgcaaggccactgataacttgagccaagaccatgctcaaggtgtaagtaagcaaactatgaatcctaagtttggcttgatggaaatcgaagttgtaagtaaggaagaaagacaaagagtatctgataagattagggatgctttagaattgccaaagactaaggtagctgctaataaagcaagttacgttatgaatcataattaa

SEQ ID NO: 14 - DNA, 888 bp, synthetic construct
  source 1..888: mol_type = other DNA
atggaacaagaacaaaagcaaactgataatacaattgatcttactcaattgcttcaactttgtcgcagacatatctgggcattgattctttggagtattggattaacattagtaggttggggaattgctaactttgtcatttcaccaaagtatacttctagtgcacaaatcttagttaaccaaaaatccaataagaatgatcctaatacagcatatataacccaacaagctaacatgcagttagttaatacctataaagatattgtaactagtcatgtaatcttgaaggatgcttctgatcgtttgactaacccagttagagtggttaagaaggctaagccagctaagtacaaaactactgataatggtagaaaagtcttggtgagaaaggctcaaccagcagtcattaaacgtgacggtaaggcatatagcgtttcagctgcgcaattagctaagagtgtttcagttgctacgcaacaacaatcacaggtattctcagtttctgctacggctgatactcctgaaaaggctaaggctgaagctaatgcagttgctagatcattcagagatcaaattcctaatatcatgaatatcgataacgttacgatcgttgcatcagctactaatggtgttcaatcatcacctaacgttaagatgtttactttagcaggatttgttattggtttagtattaacctttgcagtgatcttaattcgtgaaatgactaataccactgttcgtgatgatacttacttaactcaagatttgggtttgaccaacttaggatatgtatctcacttccatgtatcttcatcatttaagttgattaagaataataataataagccagctgctaagcgtgaacaacgcaagagacgcagagtatag

SEQ ID NO: 15 - protein, 99 aa, synthetic construct
MIVALSTDEFNREKGKKSYFNYNKRKSLLESIRYVDLVIPENNWDQKINDMHEYHIDTFVMGDDWKGKFDFIKDEGVDVVYLPRTPEISTRKIKRDLKL

SEQ ID NO: 16 - protein, 363 aa, synthetic construct
MKIALINTVNLEENGISTFILNNSYLFSKWGEDVAIIAPNKVKKALKKRIISKGIRLIELPMRDNSPQIYFWKLIKVLKKEKYDIVHVNGNSTTMSVELLAAWIAGIQVRIAHSHNTTADHTNINKLLRPIFNLTVNGRVACNIAAGKWLFHQKKFLVIRNGINLSHFHFDESLRENYRKTLKLNKDDILLGNVGKFNRQKNQVVLLDLIKQLGDNYYLVLVGSGVNFEKIKKRVDSDAFLRKHIFFTGAVSDTSGWLNAMDLFLLPSLYEGQPYTLIETTASGLDAVVSNIISSENDLVSNISFERLDSPKDWVQKIKIPIANNRELRSNSYCQKLKEKGYDTTENAKMLLKYYKKKISLYK

SEQ ID NO: 17 - protein, 271 aa, synthetic construct
MQKKVLSSNELKAIHSLELEALTVIDQICRKHSIKYTLIGGSLLGAIRHNVFIPWDDVDIAMLRDDLEKFKLICKTELPSKYFYQDMSTDPEYLYLFDKIRINNTLFKESYLAEYNINHGVFIDIFPVDNVSDKKSEDKKQFNSFIFLRHMFMAKYLSVKARKGKKKIIAGLIKYLIPNNTKKIRNKAFDIMCKYDKEKTKKVRIFPSTYAKKDVYCRKFFDEAEDHKFENHNFLISKYYEQMLVNDYGNWRELPPKDQRVTRHNLVDFKL

SEQ ID NO: 18 - protein, 487 aa, synthetic construct
MSKKSLGLNAFLNGLRSVLNLLFPLVTFPYISRVLSVSGIGIYNFSNTYIGYFILIAGLGIATYAVREGAKYRDNKEQIEEFSSEVFSINILATVIAYILLLLSLVIFKNLNNYVACILIFSIQILFTTLGTEWIYTIYEDYTYITIRSIIFKILSIILLFIFVKRPSDYLIYAAITVLASVGSNFLNFVHARSFIHIRLTLNTRWEYHLKPILTIFASSVAVTIYVYSDNTILGLMKNDYAVGIYSTSVKIYQIAQSLLSAVLTVTIPRLAMLWGQRRRREYNDVLTRVINTLGVLVLPASVGLLMLSREVVLIIAGQKFLPSVNSLRIITWAIIFSIFSWIFSDCVLIPAKRENKVLRNTLVTAVINIILNFVLIPTMSYDGTSLSTVLAELSVMIMNGYSCRDIIKPIIFKKETLKNLLESIIGCIGIVGVCLLCQWSWNSMIMVTIFSVNSSILIYGAILVLLKNKIAISMLKNAINIIKNKI

SEQ ID NO: 19 - protein, 333 aa, synthetic construct
MVDKKPIISIIIPMYNVENYIAICLNSIIQNDLKNVEVIIVNDGSTDNSRTIAERYQAKYSQIRIFDKENAGVSRARNYGLSKSTGDWIWFVDSDDAIRKGSLEYIKKMILTCYSNLDVLIFGYLRFEEKKNIDKSCSLNRIDDSKRISKFQAMGTLLDERFATFPWNKIFRRELFKKIAFPEDRIYTEDLAIIYKLYDKATHFRLENTTLYLYRIRENGLTHNLSTKKLKDSALSHYEMYTFFKANYSSLSTKLRRETLISAISFFHRLNKSQIQLYPDLIKFLNQDIYMKDCNTRYKIEIWAFKKCYPLFVTIGMIGKILRRLKNLKKGKS

SEQ ID NO: 20 - protein, 341 aa, synthetic construct
MNSLVSIVVPIYNVEKYLRKCIESLVDQTYQNIEILLIDDGSTDSSGKICDDYAETYSFVYSFHKANSGLGFTRNYGLERIKGEYVTFVDSDDYLGKNAIKRLVAGLDGKSIDTVIGGYSKVKDNGEVLYTREYTESIFRHESIYQKLFVSMLGSSPNKHNSFRPSVWNSLYSCKIIKKNSIIFASERKLISEDIVWDSDYYKFAKGVRIINSSAYYYRANPKSLSKSYRPDRFEKSIYFFMYMVDKLSKLNLANKSFTEARLRLAKTLFINVRSSLSQLEFMPIRKIIKNVREICSNADLNEVIKNYPIDKLAIRQRLFVLLIKHKFILILSILIKVQVI

SEQ ID NO: 21 - protein, 165 aa, synthetic construct
MIFVTVGTHEQPFNRLIKKVDDLVASGDIKEKVIIQIGFSTYIPKNCEAHKMMSFDEMQQALRDARIVITHGGPSSFIEALQFGKVPIVVPRQEKFHEHVNNHQVEFTKLIAERMNNIIPVYDIDDLKTTIDNYDQIAKTKNVGESSNNKQFNEKLEKIVDGLAK

SEQ ID NO: 22 - protein, 149 aa, synthetic construct
MKVCLVGSSGGHLTHLYMLKPFWQNKDRFWVTFDKEDARSKLKGEKMYGCHYPTNRNLKNLIKNTFLAIKVLRKERPDVIISSGAAVAVPFFYIGKLMGAKTVYIEVFDRYDKPTLTGKLVYPITDRFIVEWEEMKKVYPKAINLGSIF

SEQ ID NO: 23 - protein, 216 aa, synthetic construct
MVMEKLKVNPVKVHGRYVYHALKRLFDIIASAVGLILLSPLFLFLIIKIRHEDGGPAFYSQERIGKDEKPFKMWKFRSMVVNADQMIDQLEDQNEINGAMFKIKDDPRITKIGHTIRKYSLDELPQLWNVLTGDMSLVGPRPPLPSEVEEYTDYDKQRLLVMPGCTGLWQVTKRNEADFDEMAWLDIVYINHSGILEDLKLIIKTIGVVIHPNGAY

SEQ ID NO: 24 - protein, 256 aa, synthetic construct
MVLVDIHCHILPGVDDGAKDWQTSIKLAREAVADGVTHAVCTPHMLNGKYINHKKDVIRLTENFQDMLDDAKIPLTVFPGQEVRISGDLPKALDDDDILFLDVDGQYMLLEFPSDDVPAYTRDMVFELMQRGITPIVVHPERNKKILEEPTILQELIEQGCLVQITASSYMGTFGKKIEEMSRKFIKAGQCACFASDAHDLPKRQYQYSEALKKLSKEFRSDLAQQYEDNARAFVNGDNVQLDWQPLGKKKKFWLF

SEQ ID NO: 25 - protein, 261 aa, synthetic construct
MSLFKKKRGTDEAIKKGAKLITVADPKSPVTEQFRTIRTNINFMAVDHDIKSVAFTSASISEGKSAVAANVAVTYAQAGHKVLLIDADLRRPTVHRTFNLSNHVGLSTVISSTAKEVDLDEVVQDSGIADLAILPAGPTQPNPSELIGSKRMQDFISLVEDHYDMVIIDLAPVIEVSDTQELARRLDGIILVVRQGKTQKAAIKRAVEMLNFSKAKVLGFIMNDISSDNAGYGYGYGYGYGYGYGEEDAKKKKGIFSRLKK

SEQ ID NO: 26 - protein, 295 aa, synthetic construct
MEQEQKQTDNTIDLTQLLQLCRRHIWALILWSIGLTLVGWGIANFVISPKYTSSAQILVNQKSNKNDPNTAYITQQANMQLVNTYKDIVTSHVILKDASDRLTNPVRVVKKAKPAKYKTTDNGRKVLVRKAQPAVIKRDGKAYSVSAAQLAKSVSVATQQQSQVFSVSATADTPEKAKAEANAVARSFRDQIPNIMNIDNVTIVASATNGVQSSPNVKMFTLAGFVIGLVLTFAVILIREMTNTTVRDDTYLTQDLGLTNLGYVSHFHVSSSFKLIKNNNNKPAAKREQRKRRRV

SEQ ID NO: 27 - protein, 351 aa, synthetic construct
MVEKNQQDKKPMRRHHHHHRHHHRKFWRGFWIVLGIVVVIGLFVCGMVYKNLRSTTQNMYTPVAKNTKSNKGRTLDNLLNEKKPINILLLGIDTGAMGRHWKGRTDTMMMMSINPKKNTTTIVSIPRDSNAIFPDYPEYGVTKMNSAYTLGGVSETIKTLDKYYSVPIDGYIMINMGGLKKAIDQVGGIDVTSPLTFNNMGYHFEEGKTYHMNGKKALAFAQLRHGDPRQDYGRQDRDRRVIMALLKKSVSPTTLLNSNFLNSISDEMQTDLTMNQMYKIGMDYRKATDNLSQDHAQGVSKQTMNPKFGLMEIEVVSKEERQRVSDKIRDALELPKTKVAANKASYVMNHN

SEQ ID NO: 28 - DNA, 60 bp, synthetic construct
  source 1..60: mol_type = other DNA
agtctggaaacgcggaagtcagcgccctgcaccatttatggtattatattctggtaatga

SEQ ID NO: 29 - DNA, 60 bp, synthetic construct
  source 1..60: mol_type = other DNA
ataattaaatttttagaggccaggatctggtcccgccgcatccataccgccagttgttta

SEQ ID NO: 30 - DNA, 60 bp, synthetic construct
  source 1..60: mol_type = other DNA
gaagcgactgctgctgcaaaacgtctgcgacctgattatggtattatattctggtaatga

SEQ ID NO: 31 - DNA, 60 bp, synthetic construct
  source 1..60: mol_type = other DNA
ttattcgctattttccatttcctatatcatcagtaacccgtatcgtgagcatcctctctc

SEQ ID NO: 32 - DNA, 60 bp, synthetic construct
  source 1..60: mol_type = other DNA
tttcatcggtatcattacccccatgaacagaaatcttatggtattatattctggtaatga

SEQ ID NO: 33 - DNA, 59 bp, synthetic construct
  source 1..59: mol_type = other DNA
atgtcaattgactttaccccaggtatcaccgatacgcgagcgaacgtgaagcgactgct

SEQ ID NO: 34 - DNA, 25 bp, synthetic construct
  source 1..25: mol_type = other DNA
atgtcaattgactttaccccaggta

SEQ ID NO: 35 - DNA, 25 bp, synthetic construct
  source 1..25: mol_type = other DNA
ttatggtattatattctggtaatga

SEQ ID NO: 36 - DNA, 47 bp, synthetic construct
  source 1..47: mol_type = other DNA
gggtttaggattagcgataacaatgtacgaagagcaaaaaatacggc

SEQ ID NO: 37 - DNA, 47 bp, synthetic construct
  source 1..47: mol_type = other DNA
ttattcgctattttccatttcctatcttgacaaacaaatcgaaggtt

SEQ ID NO: 38 - DNA, 25 bp, synthetic construct
  source 1..25: mol_type = other DNA
tacgaagagcaaaaaatacggcgat

SEQ ID NO: 39 - DNA, 24 bp, synthetic construct
  source 1..24: mol_type = other DNA
ggaaatggaaaatagcgaataaac

SEQ ID NO: 40 - DNA, 45 bp, synthetic construct
  source 1..45: mol_type = other DNA
aaactaaaaaatggtagataaaaagtcctaatattattttataca

SEQ ID NO: 41 - DNA, 45 bp, synthetic construct
  source 1..45: mol_type = other DNA
tttctcttaccctcaatgtcttattcgctattttccatttcctat

SEQ ID NO: 42 - DNA, 25 bp, synthetic construct
  source 1..25: mol_type = other DNA
ctaatattattttatacatcattct

SEQ ID NO: 43 - DNA, 25 bp, synthetic construct
  source 1..25: mol_type = other DNA
gacattgagggtaagagaaaaaatg

SEQ ID NO: 44 - DNA, 46 bp, synthetic construct
  source 1..46: mol_type = other DNA
aaatgatggtaatggagaaactaaagctaatgccacaaatctgcag

SEQ ID NO: 45 - DNA, 46 bp, synthetic construct
  source 1..46: mol_type = other DNA
ctcaatatattatagacctttataattaaatttttagaggccagga

SEQ ID NO: 46 - DNA, 19 bp, synthetic construct
  source 1..19: mol_type = other DNA
gctaatgccacaaatctgc

SEQ ID NO: 47 - DNA, 23 bp, synthetic construct
  source 1..23: mol_type = other DNA
aggtctataatatattgagggga

SEQ ID NO: 48 - protein, 321 aa, synthetic construct
MKRACFIIPYFGKLPNYFQLFLNSCAPNKKFDWLIITNDNRGFSYPKNVKKIFMEWNEFKRFAQKKFKEKLALEYPKKLCDFKPTYGYLFEDLIRQYSYWGYCDIDTIMGNLDEQLPLSFLNKYDKIFSLGHMVLFKNSFEINRAFLKPVNKEYYYKKALTSDKIEVFDETGNGKKNIDTIFVKNGYNVFHADWSYNPRVTPTKFKNVIYDYYTDDFYTENYKKSICIWDGHNIVRYVINNNNLKKESFLYVHLQQRKMKLGSNVLKAKAFSIIPNEFNLLDLPVDVSKNYIKKLKREDLNPHYFRIMWKWKIANKLKNGR

SEQ ID NO: 49 - protein, 387 aa, synthetic construct
MKIRLERERLYCLGLALFLVGQLLGHTLLPVPLHGRYFLIYLGIFISIFSFIIDFRELYYAVNRLTLEKIEVIIFIIILTIVSIISFKHNYSYALIVNIIFILSAYHIRFEKILKTFFVVACSVLLIMLLAYILGLVGDGQVLQGRKTFGYRMPTDLVQLIVYITLSKIYLNLMKGRNNTSLYLLIFVIAIITLVESSSRLGSLTLLLLIPYTIFLKRKIFKSDFQISKFTQSILKNLFFIGALLSYLVTELFIRYPNNSVLEFINQITSARLTNNRMGIEFWGYSIWGQDIYTNISSFFKGWFYIDNSFYVFLLSYGLVLLILVGLGYRYLVQKCLKKQEYIVPFVLLAIVLDSLIDQHFYSLEYNIFLLTPFSTLITYTNEEGLK

SEQ ID NO: 50 - protein, 239 aa, synthetic construct
MSIKDKIKTILFGYKATEETYLTHLRNSGVKLGTNIKIFRPFNTTIDVQNPHLLTIGNDVQITGPVTILTHDYSWSVLKKKYGIIYGNQRKTVIGNNVFIGWGVTILGGSHIGDNVIIGANSVVSGNVDSNSVYAGNPARKLMTLEEYRDKREKRQLKEAVEYVLEYKKRFKTYPPEEKMDEYFFLFRPSKIFNEYRAQLELMRNFDKSLKKLNNSNTQFLSYKEFLNYCKKQKMVERK

SEQ ID NO: 51 - protein, 103 aa, synthetic construct
MGIMYSSITAVEKINIGNHVNIANNVVIVDHDHFVDKKGVHGNLITAPVNIEDHVWIGANVTITKGVNIGEGAVIAAGAVVTHDVPAHTVVGGIPANKIKKID

SEQ ID NO: 52 - DNA, 966 bp, synthetic construct
  source 1..966: mol_type = other DNA
ttatctaccattttttagtttattcgctattttccatttccacataattctaaaataatgaggattcaaatcttcccgttttagttttttaatataattcttcgacacatcaactggtaaatctaacaaattaaattcattcggtattatactaaacgcttttgcctttaatacatttgaacctaatttcatttttctctgctgcaaatggacatataaaaagctttccttttttaaattattattgttaattacatatctaactatattatgtccatcccaaatgcatatagatttcttataattttcggtatagaaatcatctgtataataatcatatattacatttttgaattttgttggtgtaacacgtggattatatgaccagtctgcatgaaaaacgttatatccatttttcacaaagatagtatctatatttttctttccatttccagtttcatcaaatacttcaattttatctgaagttaaggctttcttatagtaatattctttatttacaggctttaaaaaagctctatttatctcaaaactgtttttaaataaaaccatatgtcctagggagaatattttatcgtatttatttaaaaaagataatggtaattgctcatctagatttcccataatagtatctatatcacaatagccccagtaagaatattgtctaattaaatcctcaaacagatatccatatgtaggtttaaaatcacacaatttttttggatattccaaagctaatttttctttaaactttttctgtgcaaatcgtttaaattcattccattccataaagattttcttaacatttttaggatatgaaaatcctctattatcattcgttataattagccaatcaaatttcttatttggtgcacaactattcaaaaataattggaaataattgggaagttttccaaaatatggaattataaaacatgctcttttcat

SEQ ID NO: 53 - DNA, 1164 bp, synthetic construct
  source 1..1164: mol_type = other DNA
tcattttaatccttcttcattagtgtacgttatcaatgttgagaatggcgttaataagaatatgttatattctaaggaataaaagtgttgatctattaaactatctaaaactatagcaagtaaaacaaatggaactatatattcttgtttctttaaacacttttggactaaatatctataacctaatcctacaagaattaataatactaatccatacgatagcaaaaatacataaaaactattgtcaatataaaaccagcctttgaaaaaagaagaaatattagtataaatatcttgcccccagatagaatatccccaaaattcaatccccattctattatttgttaatctagccgaagtaatttgattaataaattcaagcaccgaattatttggatatctgataaaaagttccgttactaaatacgataataatgcacctataaaaaagagatttttaagaattgattgtgtaaatttagaaatttgaaaatcagatttaaaaatttttctttttaggaagatagtatacggtataagtaaaagtaatgtgagacttcctagtctagaactactttccactaaagttattattgctataacaaatattaataagtataaggaagtattattacgtcctttcatcaaatttaaatagatcttggataaagtaatatatactatcagctgaactaaatccgttggcattctatatccaaacgtctttcttccttgaagtacctgtccatctccaaccaaacctagaatataagctaataacattattagcaacacactacaggcaactacaaaaaaagtcttcaatattttctcaaagcgtatgtgataggcacttaaaataaagataatattaacaattaaagcataactataattgtgcttaaaagaaattatagagacaatagttaaaataattataaaaataattacttctattttctcaagggtaagcctatttactgcataatataattcacgaaaatctataataaaactaaatatggaaataaagatgcccaaatatattaaaaaatatcttccatgtaatggtacaggtaataatgtatgtcctaagagctgaccaactaaaaataaggctaatcccagacaatacaatctctcccgctcaagtcttattttcat

SEQ ID NO: 54 - DNA, 720 bp, synthetic construct
  source 1..720: mol_type = other DNA
tcatttacgttccaccatcttttgctttttacaataattcaaaaattctttatatgacaaaaactgagtattggaattattcaatttttttaagcttttatcaaagtttctcattaattctaattgagccctatactcattaaatattttagaaggtctaaataaaaagaaatactcatccatcttttcttctggtggataagtcttaaatcttttcttgtactctaaaacgtattctactgcctcttttaattggcgtttctctcttttatctctatattcttcaagagtcattagttttcgagcgggatttcctgcatatacagaattagaatcaacatttccacttacaacactattggcaccaattattacattatcaccaatatgtgatccacctagaattgtaacgccccatcctataaatacgttattgcctattacagttttacgttgatttccataaataattccatattttttcttcaacacagaccaactgtaatcatgcgttaatatagttaccggacccgttatttgaacatcatttccaattgtcaaaagatgcggattttgtacatcaattgttgtattgaatgggcgaaaaatttttatattagtacctaatttaactccgctatttcttaaatgtgttaagtatgtttcttcagtagccttatatccaaataaaatagtcttaattttgtcttttatgctcat

SEQ ID NO: 55 - DNA, 312 bp, synthetic construct
  source 1..312: mol_type = other DNA
ttaatctatttttttgattttattagcggggatgcctccaactactgtatgagcaggaacatcatgcgtcacaacggctccagctgcaatcacagcaccttctccaatattaacacccttagtaatagtaacatttgcaccaatccacacatgatcttcaatattaacaggtgcagtaattaagttcccatgaaccccttttttatcaacaaaatgatcatgatctacaatcactacattattagcaatatttacgtgattacctatatttatcttctcaactgcagtaattgaagaatacataatccccaa